European Patent Application EP 4 685 231 A1, published January 28, 2026. Title: 幽门螺杆菌岩藻糖基转移酶突变体. Applicant: 北京睿脉医药科技有限公司. The sequence listing filed with the application follows.

SEQUENCE LISTING (10 sequences)

SEQ ID NO: 1 - protein, 411 aa, Helicobacter pylori
MFQPLLDAFIESASIEKMVSKSPPPPLKIAVANWWGDEEIKEFKKSVLYFILSQRYAITLHQNPNESSDLVFSNPLGAARKILSYQNTKRVFYTGENESPNFNLFDYAIGFDELDFNDRYLRMPLYYAHLHYEAELVNDTTAPYKLKDNSLYALKKPSHHFKENHPNLCAVVNDESDLLKRGFASFVASNANAPMRNAFYDALNSIEPVTGGGSVRNTLGYKVGNKSEFLSQYKFNLCFENSQGYGYVTEKILDAYFSHTIPIYWGSPSVAKDFNPKSFVNVHDFNNFDEAIDYIKYLHTHPNAYLDMLYENPLNTLDGKAYFYQDLSFKKILDFFKTILENDTIYHNNPFIFYRDLHEPLISIDDLRVNYDDLRVNYDDLRVNYDDLRVNYDDLRVNYDDLRVNHHHHHH

SEQ ID NO: 2 - DNA, 1233 bp, Helicobacter pylori
  source 1..1233: mol_type = other DNA
atgtttcagccgctgctggatgcgtttattgaaagcgcgagcattgaaaaaatggtgagcaaaagcccgccgccgccgctgaaaattgcggtggcgaactggtggggcgatgaagaaattaaagaatttaaaaaaagcgtgctgtattttattctgagtcagcgctatgcgattaccctgcatcagaacccgaacgaaagcagcgatctggtgtttagcaacccgctgggcgcggcgcgcaaaattctgagctatcagaacaccaaacgcgtgttttataccggcgaaaacgaaagcccgaactttaacctgtttgattatgcgattggctttgatgaactggattttaacgatcgctatctgcgcatgccgctgtattatgcgcatctgcattatgaagcggaactggtgaacgataccaccgcgccgtataaactgaaagataacagcctgtatgcgctgaaaaaaccgagccatcattttaaagaaaaccatccgaacctgtgcgcggtggtgaacgatgaaagcgatctgctgaaacgcggctttgcgagctttgtggcgagcaacgcgaacgcgccgatgcgcaacgcgttttatgatgcgctgaacagcattgaaccggtgaccggcggcggcagcgtgcgcaacaccctgggctataaagtgggcaacaaaagcgaatttctgagtcagtataaatttaacctgtgctttgaaaacagccaaggctatggctatgtgaccgaaaagattctggacgcgtattttagccataccattccgatttattggggcagcccgagcgtggcgaaagattttaacccgaaaagctttgtgaacgtgcatgattttaacaactttgatgaagcgattgattatattaaatatctgcatacccatccgaacgcgtatctggatatgctgtatgaaaacccgctgaacaccctggatggcaaagcatatttttatcaagatctgagcttcaagaaaatactggattttttcaaaaccattctggaaaacgataccatttatcataacaacccgtttattttttatcgcgatctgcatgaaccgctgattagcattgacgacctgagggtgaattatgacgaccttcgcgtcaactacgatgatcttcgcgtgaattatgacgacctccgcgtgaactatgacgatttacgcgtcaattacgatgacttacgcgtaaaccatcatcaccatcatcac

SEQ ID NO: 3 - protein, 411 aa, synthetic construct
  REGION 1..411: note = P64S
MFQPLLDAFIESASIEKMVSKSPPPPLKIAVANWWGDEEIKEFKKSVLYFILSQRYAITLHQNSNESSDLVFSNPLGAARKILSYQNTKRVFYTGENESPNFNLFDYAIGFDELDFNDRYLRMPLYYAHLHYEAELVNDTTAPYKLKDNSLYALKKPSHHFKENHPNLCAVVNDESDLLKRGFASFVASNANAPMRNAFYDALNSIEPVTGGGSVRNTLGYKVGNKSEFLSQYKFNLCFENSQGYGYVTEKILDAYFSHTIPIYWGSPSVAKDFNPKSFVNVHDFNNFDEAIDYIKYLHTHPNAYLDMLYENPLNTLDGKAYFYQDLSFKKILDFFKTILENDTIYHNNPFIFYRDLHEPLISIDDLRVNYDDLRVNYDDLRVNYDDLRVNYDDLRVNYDDLRVNHHHHHH

SEQ ID NO: 4 - DNA, 1233 bp, synthetic construct
  misc_feature 1..1233: note = P64S
  source 1..1233: mol_type = other DNA
atgtttcagccgctgctggatgcgtttattgaaagcgcgagcattgaaaaaatggtgagcaaaagcccgccgccgccgctgaaaattgcggtggcgaactggtggggcgatgaagaaattaaagaatttaaaaaaagcgtgctgtattttattctgagtcagcgctatgcgattaccctgcatcagaactcgaacgaaagcagcgatctggtgtttagcaacccgctgggcgcggcgcgcaaaattctgagctatcagaacaccaaacgcgtgttttataccggcgaaaacgaaagcccgaactttaacctgtttgattatgcgattggctttgatgaactggattttaacgatcgctatctgcgcatgccgctgtattatgcgcatctgcattatgaagcggaactggtgaacgataccaccgcgccgtataaactgaaagataacagcctgtatgcgctgaaaaaaccgagccatcattttaaagaaaaccatccgaacctgtgcgcggtggtgaacgatgaaagcgatctgctgaaacgcggctttgcgagctttgtggcgagcaacgcgaacgcgccgatgcgcaacgcgttttatgatgcgctgaacagcattgaaccggtgaccggcggcggcagcgtgcgcaacaccctgggctataaagtgggcaacaaaagcgaatttctgagtcagtataaatttaacctgtgctttgaaaacagccaaggctatggctatgtgaccgaaaagattctggacgcgtattttagccataccattccgatttattggggcagcccgagcgtggcgaaagattttaacccgaaaagctttgtgaacgtgcatgattttaacaactttgatgaagcgattgattatattaaatatctgcatacccatccgaacgcgtatctggatatgctgtatgaaaacccgctgaacaccctggatggcaaagcatatttttatcaagatctgagcttcaagaaaatactggattttttcaaaaccattctggaaaacgataccatttatcataacaacccgtttattttttatcgcgatctgcatgaaccgctgattagcattgacgacctgagggtgaattatgacgaccttcgcgtcaactacgatgatcttcgcgtgaattatgacgacctccgcgtgaactatgacgatttacgcgtcaattacgatgacttacgcgtaaaccatcatcaccatcatcac

SEQ ID NO: 5 - protein, 411 aa, synthetic construct
  REGION 1..411: note = A108V
MFQPLLDAFIESASIEKMVSKSPPPPLKIAVANWWGDEEIKEFKKSVLYFILSQRYAITLHQNPNESSDLVFSNPLGAARKILSYQNTKRVFYTGENESPNFNLFDYVIGFDELDFNDRYLRMPLYYAHLHYEAELVNDTTAPYKLKDNSLYALKKPSHHFKENHPNLCAVVNDESDLLKRGFASFVASNANAPMRNAFYDALNSIEPVTGGGSVRNTLGYKVGNKSEFLSQYKFNLCFENSQGYGYVTEKILDAYFSHTIPIYWGSPSVAKDFNPKSFVNVHDFNNFDEAIDYIKYLHTHPNAYLDMLYENPLNTLDGKAYFYQDLSFKKILDFFKTILENDTIYHNNPFIFYRDLHEPLISIDDLRVNYDDLRVNYDDLRVNYDDLRVNYDDLRVNYDDLRVNHHHHHH

SEQ ID NO: 6 - DNA, 1233 bp, synthetic construct
  misc_feature 1..1233: note = A108V
  source 1..1233: mol_type = other DNA
atgtttcagccgctgctggatgcgtttattgaaagcgcgagcattgaaaaaatggtgagcaaaagcccgccgccgccgctgaaaattgcggtggcgaactggtggggcgatgaagaaattaaagaatttaaaaaaagcgtgctgtattttattctgagtcagcgctatgcgattaccctgcatcagaacccgaacgaaagcagcgatctggtgtttagcaacccgctgggcgcggcgcgcaaaattctgagctatcagaacaccaaacgcgtgttttataccggcgaaaacgaaagcccgaactttaacctgtttgattatgtgattggctttgatgaactggattttaacgatcgctatctgcgcatgccgctgtattatgcgcatctgcattatgaagcggaactggtgaacgataccaccgcgccgtataaactgaaagataacagcctgtatgcgctgaaaaaaccgagccatcattttaaagaaaaccatccgaacctgtgcgcggtggtgaacgatgaaagcgatctgctgaaacgcggctttgcgagctttgtggcgagcaacgcgaacgcgccgatgcgcaacgcgttttatgatgcgctgaacagcattgaaccggtgaccggcggcggcagcgtgcgcaacaccctgggctataaagtgggcaacaaaagcgaatttctgagtcagtataaatttaacctgtgctttgaaaacagccaaggctatggctatgtgaccgaaaagattctggacgcgtattttagccataccattccgatttattggggcagcccgagcgtggcgaaagattttaacccgaaaagctttgtgaacgtgcatgattttaacaactttgatgaagcgattgattatattaaatatctgcatacccatccgaacgcgtatctggatatgctgtatgaaaacccgctgaacaccctggatggcaaagcatatttttatcaagatctgagcttcaagaaaatactggattttttcaaaaccattctggaaaacgataccatttatcataacaacccgtttattttttatcgcgatctgcatgaaccgctgattagcattgacgacctgagggtgaattatgacgaccttcgcgtcaactacgatgatcttcgcgtgaattatgacgacctccgcgtgaactatgacgatttacgcgtcaattacgatgacttacgcgtaaaccatcatcaccatcatcac

SEQ ID NO: 7 - protein, 411 aa, synthetic construct
  REGION 1..411: note = D139E
MFQPLLDAFIESASIEKMVSKSPPPPLKIAVANWWGDEEIKEFKKSVLYFILSQRYAITLHQNPNESSDLVFSNPLGAARKILSYQNTKRVFYTGENESPNFNLFDYAIGFDELDFNDRYLRMPLYYAHLHYEAELVNETTAPYKLKDNSLYALKKPSHHFKENHPNLCAVVNDESDLLKRGFASFVASNANAPMRNAFYDALNSIEPVTGGGSVRNTLGYKVGNKSEFLSQYKFNLCFENSQGYGYVTEKILDAYFSHTIPIYWGSPSVAKDFNPKSFVNVHDFNNFDEAIDYIKYLHTHPNAYLDMLYENPLNTLDGKAYFYQDLSFKKILDFFKTILENDTIYHNNPFIFYRDLHEPLISIDDLRVNYDDLRVNYDDLRVNYDDLRVNYDDLRVNYDDLRVNHHHHHH

SEQ ID NO: 8 - DNA, 1233 bp, synthetic construct
  misc_feature 1..1233: note = D139E
  source 1..1233: mol_type = other DNA
atgtttcagccgctgctggatgcgtttattgaaagcgcgagcattgaaaaaatggtgagcaaaagcccgccgccgccgctgaaaattgcggtggcgaactggtggggcgatgaagaaattaaagaatttaaaaaaagcgtgctgtattttattctgagtcagcgctatgcgattaccctgcatcagaacccgaacgaaagcagcgatctggtgtttagcaacccgctgggcgcggcgcgcaaaattctgagctatcagaacaccaaacgcgtgttttataccggcgaaaacgaaagcccgaactttaacctgtttgattatgcgattggctttgatgaactggattttaacgatcgctatctgcgcatgccgctgtattatgcgcatctgcattatgaagcggaactggtgaacgaaaccaccgcgccgtataaactgaaagataacagcctgtatgcgctgaaaaaaccgagccatcattttaaagaaaaccatccgaacctgtgcgcggtggtgaacgatgaaagcgatctgctgaaacgcggctttgcgagctttgtggcgagcaacgcgaacgcgccgatgcgcaacgcgttttatgatgcgctgaacagcattgaaccggtgaccggcggcggcagcgtgcgcaacaccctgggctataaagtgggcaacaaaagcgaatttctgagtcagtataaatttaacctgtgctttgaaaacagccaaggctatggctatgtgaccgaaaagattctggacgcgtattttagccataccattccgatttattggggcagcccgagcgtggcgaaagattttaacccgaaaagctttgtgaacgtgcatgattttaacaactttgatgaagcgattgattatattaaatatctgcatacccatccgaacgcgtatctggatatgctgtatgaaaacccgctgaacaccctggatggcaaagcatatttttatcaagatctgagcttcaagaaaatactggattttttcaaaaccattctggaaaacgataccatttatcataacaacccgtttattttttatcgcgatctgcatgaaccgctgattagcattgacgacctgagggtgaattatgacgaccttcgcgtcaactacgatgatcttcgcgtgaattatgacgacctccgcgtgaactatgacgatttacgcgtcaattacgatgacttacgcgtaaaccatcatcaccatcatcac

SEQ ID NO: 9 - protein, 411 aa, synthetic construct
  REGION 1..411: note = N167Q
MFQPLLDAFIESASIEKMVSKSPPPPLKIAVANWWGDEEIKEFKKSVLYFILSQRYAITLHQNPNESSDLVFSNPLGAARKILSYQNTKRVFYTGENESPNFNLFDYAIGFDELDFNDRYLRMPLYYAHLHYEAELVNDTTAPYKLKDNSLYALKKPSHHFKENHPQLCAVVNDESDLLKRGFASFVASNANAPMRNAFYDALNSIEPVTGGGSVRNTLGYKVGNKSEFLSQYKFNLCFENSQGYGYVTEKILDAYFSHTIPIYWGSPSVAKDFNPKSFVNVHDFNNFDEAIDYIKYLHTHPNAYLDMLYENPLNTLDGKAYFYQDLSFKKILDFFKTILENDTIYHNNPFIFYRDLHEPLISIDDLRVNYDDLRVNYDDLRVNYDDLRVNYDDLRVNYDDLRVNHHHHHH

SEQ ID NO: 10 - DNA, 1233 bp, synthetic construct
  misc_feature 1..1233: note = N167Q
  source 1..1233: mol_type = other DNA
atgtttcagccgctgctggatgcgtttattgaaagcgcgagcattgaaaaaatggtgagcaaaagcccgccgccgccgctgaaaattgcggtggcgaactggtggggcgatgaagaaattaaagaatttaaaaaaagcgtgctgtattttattctgagtcagcgctatgcgattaccctgcatcagaacccgaacgaaagcagcgatctggtgtttagcaacccgctgggcgcggcgcgcaaaattctgagctatcagaacaccaaacgcgtgttttataccggcgaaaacgaaagcccgaactttaacctgtttgattatgcgattggctttgatgaactggattttaacgatcgctatctgcgcatgccgctgtattatgcgcatctgcattatgaagcggaactggtgaacgataccaccgcgccgtataaactgaaagataacagcctgtatgcgctgaaaaaaccgagccatcattttaaagaaaaccatccgcagctgtgcgcggtggtgaacgatgaaagcgatctgctgaaacgcggctttgcgagctttgtggcgagcaacgcgaacgcgccgatgcgcaacgcgttttatgatgcgctgaacagcattgaaccggtgaccggcggcggcagcgtgcgcaacaccctgggctataaagtgggcaacaaaagcgaatttctgagtcagtataaatttaacctgtgctttgaaaacagccaaggctatggctatgtgaccgaaaagattctggacgcgtattttagccataccattccgatttattggggcagcccgagcgtggcgaaagattttaacccgaaaagctttgtgaacgtgcatgattttaacaactttgatgaagcgattgattatattaaatatctgcatacccatccgaacgcgtatctggatatgctgtatgaaaacccgctgaacaccctggatggcaaagcatatttttatcaagatctgagcttcaagaaaatactggattttttcaaaaccattctggaaaacgataccatttatcataacaacccgtttattttttatcgcgatctgcatgaaccgctgattagcattgacgacctgagggtgaattatgacgaccttcgcgtcaactacgatgatcttcgcgtgaattatgacgacctccgcgtgaactatgacgatttacgcgtcaattacgatgacttacgcgtaaaccatcatcaccatcatcac